European Patent Application EP 4 722 237 A1, published April 8, 2026. Title: 检测胰岛素或其类似物的生物学活性的方法及试剂盒. Applicant: 广东东阳光药业股份有限公司. Application CN 202310620396.9. The sequence listing filed with the application follows.

SEQUENCE LISTING (7 sequences)

SEQ ID NO: 1 - DNA, 82 bp, synthetic construct
  source 1..82: mol_type = other DNA
ggtacctgagctcgctagcgctgcttccgggaagggctgctgcttccgggaagggctgctgcttccgggaagggctagatct

SEQ ID NO: 2 - DNA, 115 bp, synthetic construct
  source 1..115: mol_type = other DNA
ggtacctgagctcgctagctgtgtggacttcttggaattaagggacttttgtgtggacttcttggaattaagggacttttgtgtggacttcttggaattaagggactttagatct

SEQ ID NO: 3 - DNA, 79 bp, synthetic construct
  source 1..79: mol_type = other DNA
ggtacctgagctcgctagcctgatttccccgaaatgactgatttccccgaaatgactgatttccccgaaatgaagatct

SEQ ID NO: 4 - protein, 1382 aa, synthetic construct [sequence omitted]

SEQ ID NO: 5 - protein, 591 aa, synthetic construct
MEDAKNIKKGPAPFYPLEDGTAGEQLHKAMKRYALVPGTIAFTDAHIEVDITYAEYFEMSVRLAEAMKRYGLNTNHRIVVCSENSLQFFMPVLGALFIGVAVAPANDIYNERELLNSMGISQPTVVFVSKKGLQKILNVQKKLPIIQKIIIMDSKTDYQGFQSMYTFVTSHLPPGFNEYDFVPESFDRDKTIALIMNSSGSTGLPKGVALPHRTACVRFSHARDPIFGNQIIPDTAILSVVPFHHGFGMFTTLGYLICGFRVVLMYRFEEELFLRSLQDYKIQSALLVPTLFSFFAKSTLIDKYDLSNLHEIASGGAPLSKEVGEAVAKRFHLPGIRQGYGLTETTSAILITPEGDDKPGAVGKVVPFFEAKVVDLDTGKTLGVNQRGELCVRGPMIMSGYVNNPEATNALIDKDGWLHSGDIAYWDEDEHFFIVDRLKSLIKYKGYQVAPAELESILLQHPNIFDAGVAGLPDDDAGELPAAVVVLEHGKTMTEKEIVDYVASQVTTAKKLRGGVVFVDEVPKGLTGKLDARKIREILIKAKKGGKIAVNSHGFPPEVEEQAAGTLPMSCAQESGMDRHPAACASARINV

SEQ ID NO: 6 - DNA, 4149 bp, synthetic construct
  source 1..4149: mol_type = other DNA
atgggcaccgggggccggcggggggcggcggccgcgccgctgctggtggcggtggccgcgctgctactgggcgccgcgggccacctgtaccccggagaggtgtgtcccggcatggatatccggaacaacctcactaggttgcatgagctggagaattgctctgtcatcgaaggacacttgcagatactcttgatgttcaaaacgaggcccgaagatttccgagacctcagtttccccaaactcatcatgatcactgattacttgctgctcttccgggtctatgggctcgagagcctgaaggacctgttccccaacctcacggtcatccggggatcacgactgttctttaactacgcgctggtcatcttcgagatggttcacctcaaggaactcggcctctacaacctgatgaacatcacccggggttctgtccgcatcgagaagaacaatgagctctgttacttggccactatcgactggtcccgtatcctggattccgtggaggataattacatcgtgttgaacaaagatgacaacgaggagtgtggagacatctgtccgggtaccgcgaagggcaagaccaactgccccgccaccgtcatcaacgggcagtttgtcgaacgatgttggactcatagtcactgccagaaagtttgcccgaccatctgtaagtcacacggctgcaccgccgaaggcctctgttgccacagcgagtgcctgggcaactgttctcagcccgacgaccccaccaagtgcgtggcctgccgcaacttctacctggacggcaggtgtgtggagacctgcccgcccccgtactaccacttccaggactggcgctgtgtgaacttcagcttctgccaggacctgcaccacaaatgcaagaactcgcggaggcagggctgccaccagtacgtcattcacaacaacaagtgcatccctgagtgtccctccgggtacacgatgaattccagcaacttgctgtgcaccccatgcctgggtccctgtcccaaggtgtgccacctcctagaaggcgagaagaccatcgactcggtgacgtctgcccaggagctccgaggatgcaccgtcatcaacgggagtctgatcatcaacattcgaggaggcaacaatctggcagctgagctagaagccaacctcggcctcattgaagaaatttcagggtatctaaaaatccgccgatcctacgctctggtgtcactttccttcttccggaagttacgtctgattcgaggagagaccttggaaattgggaactactccttctatgccttggacaaccagaacctaaggcagctctgggactggagcaaacacaacctcaccatcactcaggggaaactcttcttccactataaccccaaactctgcttgtcagaaatccacaagatggaagaagtttcaggaaccaaggggcgccaggagagaaacgacattgccctgaagaccaatggggaccaggcatcctgtgaaaatgagttacttaaattttcttacattcggacatcttttgacaagatcttgctgagatgggagccgtactggccccccgacttccgagacctcttggggttcatgctgttctacaaagaggccccttatcagaatgtgacggagttcgacgggcaggatgcatgtggttccaacagttggacggtggtagacattgacccacccctgaggtccaacgaccccaaatcacagaaccacccagggtggctgatgcggggtctcaagccctggacccagtatgccatctttgtgaagaccctggtcaccttttcggatgaacgccggacctatggggccaagagtgacatcatttatgtccagacagatgccaccaacccctctgtgcccctggatccaatctcagtgtctaactcatcatcccagattattctgaagtggaaaccaccctccgaccccaatggcaacatcacccactacctggttttctgggagaggcaggcggaagacagtgagctgttcgagctggattattgcctcaaagggctgaagctgccctcgaggacctggtctccaccattcgagtctgaagattctcagaagcacaaccagagtgagtatgaggattcggccggcgaatgctgctcctgtccaaagacagactctcagatcctgaaggagctggaggagtcctcgtttaggaagacgtttgaggattacctgcacaacgtggttttcgtccccagaaaaacctcttcaggcactggtgccgaggaccctaggccatctcggaaacgcaggtcccttggcgatgttgggaatgtgacggtggccgtgcccacggtggcagctttccccaacacttcctcgaccagcgtgcccacgagtccggaggagcacaggccttttgagaaggtggtgaacaaggagtcgctggtcatctccggcttgcgacacttcacgggctatcgcatcgagctgcaggcttgcaaccaggacacccctgaggaacggtgcagtgtggcagcctacgtcagtgcgaggaccatgcctgaagccaaggctgatgacattgttggccctgtgacgcatgaaatctttgagaacaacgtcgtccacttgatgtggcaggagccgaaggagcccaatggtctgatcgtgctgtatgaagtgagttatcggcgatatggtgatgaggagctgcatctctgcgtctcccgcaagcacttcgctctggaacggggctgcaggctgcgtgggctgtcaccggggaactacagcgtgcgaatccgggccacctcccttgcgggcaacggctcttggacggaacccacctatttctacgtgacagactatttagacgtcccgtcaaatattgcaaaaattatcatcggccccctcatctttgtctttctcttcagtgttgtgattggaagtatttatctattcctgagaaagaggcagccagatgggccgctgggaccgctttacgcttcttcaaaccctgagtatctcagtgccagtgatgtgtttccatgctctgtgtacgtgccggacgagtgggaggtgtctcgagagaagatcaccctccttcgagagctggggcagggctccttcggcatggtgtatgagggcaatgccagggacatcatcaagggtgaggcagagacccgcgtggcggtgaagacggtcaacgagtcagccagtctccgagagcggattgagttcctcaatgaggcctcggtcatgaagggcttcacctgccatcacgtggtgcgcctcctgggagtggtgtccaagggccagcccacgctggtggtgatggagctgatggctcacggagacctgaagagctacctccgttctctgcggccagaggctgagaataatcctggccgccctccccctacccttcaagagatgattcagatggcggcagagattgctgacgggatggcctacctgaacgccaagaagtttgtgcatcgggacctggcagcgagaaactgcatggtcgcccatgattttactgtcaaaattggagactttggaatgaccagagacatctatgaaacggattactaccggaaagggggcaagggtctgctccctgtacggtggatggcaccggagtccctgaaggatggggtcttcaccacttcttctgacatgtggtcctttggcgtggtcctttgggaaatcaccagcttggcagaacagccttaccaaggcctgtctaatgaacaggtgttgaaatttgtcatggatggagggtatctggatcaacccgacaactgtccagagagagtcactgacctcatgcgcatgtgctggcaattcaaccccaagatgaggccaaccttcctggagattgtcaacctgctcaaggacgacctgcaccccagctttccagaggtgtcgttcttccacagcgaggagaacaaggctcccgagagtgaggagctggagatggagtttgaggacatggagaatgtgcccctggaccgttcctcgcactgtcagagggaggaggcggggggccgggatggagggtcctcgctgggtttcaagcggagctacgaggaacacatcccttacacacacatgaacggaggcaagaaaaacgggcggattctgaccttgcctcggtccaatccttcctaa

SEQ ID NO: 7 - DNA, 1776 bp, synthetic construct
  source 1..1776: mol_type = other DNA
atggaagatgccaaaaacattaagaagggcccagcgccattctacccactcgaagacgggaccgccggcgagcagctgcacaaagccatgaagcgctacgccctggtgcccggcaccatcgcctttaccgacgcacatatcgaggtggacattacctacgccgagtacttcgagatgagcgttcggctggcagaagctatgaagcgctatgggctgaatacaaaccatcggatcgtggtgtgcagcgagaatagcttgcagttcttcatgcccgtgttgggtgccctgttcatcggtgtggctgtggccccagctaacgacatctacaacgagcgcgagctgctgaacagcatgggcatcagccagcccaccgtcgtattcgtgagcaagaaagggctgcaaaagatcctcaacgtgcaaaagaagctaccgatcatacaaaagatcatcatcatggatagcaagaccgactaccagggcttccaaagcatgtacaccttcgtgacttcccatttgccacccggcttcaacgagtacgacttcgtgcccgagagcttcgaccgggacaaaaccatcgccctgatcatgaacagtagtggcagtaccggattgcccaagggcgtagccctaccgcaccgcaccgcttgtgtccgattcagtcatgcccgcgaccccatcttcggcaaccagatcatccccgacaccgctatcctcagcgtggtgccatttcaccacggcttcggcatgttcaccacgctgggctacttgatctgcggctttcgggtcgtgctcatgtaccgcttcgaggaggagctattcttgcgcagcttgcaagactataagattcaatctgccctgctggtgcccacactatttagcttcttcgctaagagcactctcatcgacaagtacgacctaagcaacttgcacgagatcgccagcggcggggcgccgctcagcaaggaggtaggtgaggccgtggccaaacgcttccacctaccaggcatccgccagggctacggcctgacagaaacaaccagcgccattctgatcacccccgaaggggacgacaagcctggcgcagtaggcaaggtggtgcccttcttcgaggctaaggtggtggacttggacaccggtaagacactgggtgtgaaccagcgcggcgagctgtgcgtccgtggccccatgatcatgagcggctacgttaacaaccccgaggctacaaacgctctcatcgacaaggacggctggctgcacagcggcgacatcgcctactgggacgaggacgagcacttcttcatcgtggaccggctgaagagcctgatcaaatacaagggctaccaggtagccccagccgaactggagagcatcctgctgcaacaccccaacatcttcgacgccggggtcgccggcctgcccgacgacgatgccggcgagctgcccgccgcagtcgtcgtgctggaacacggtaaaaccatgaccgagaaggagatcgtggactatgtggccagccaggttacaaccgccaagaagctgcgcggtggtgttgtgttcgtggacgaggtgcctaaaggactgaccggcaagttggacgcccgcaagatccgcgagattctcattaaggccaagaagggcggcaagatcgccgtgaattctcacggcttccctcccgaggtggaggagcaggccgccggcaccctgcccatgagctgcgcccaggagagcggcatggatagacaccctgctgcttgcgccagcgccaggatcaacgtctaa